European Patent Application EP 4 148 128 A1, published March 15, 2023. Title: Polypeptides with transpositional activity. Applicant: Paul-Ehrlich-Institut, Bundesinstitut für Impfstoffe und biomedizinische Arzneimittel. The sequence listing filed with the application follows.

SEQUENCE LISTING (22 sequences)

SEQ ID NO: 1 - protein, 340 aa, human
MGKSKEISQDLRKKIVDLHKSGSSLGAISKRLKVPRSSVQTIVRKYKHHGTTQPSYRSGRRRVLSPRDERTLVRKVQINPRTTAKDLVKMLEETGTKVSISTVKRVLYRHNLKGRSARKKPLLQNRHKKARLRFATAHGDKDRTFWRNVLWSDETKIELFGHNDHRYVWRKKGEACKPKNTIPTVKHGGGSIMLWGCFAAGGTGALHKIDGIMRKENYVDILKQHLKTSVRKLKLGRKWVFQMDNDPKHTSKVVAKWLKDNKVKVLEWPSQSPDLNPIENLWAELKKRVRARRPTNLTQLHQLCQEEWAKIHPTYCGKLVEGYPKRLTQVKQFKGNATKY

SEQ ID NO: 2 - protein, 339 aa, human
MGKSKEISQDIRKRIVDLHKSGSSLVTISRCLKVPHSSVQTNLRNYKQHGNVQPSYRSGRRRILCPRDERAMVRTVCINPRTKAKDLVKMLAEAGKRVSLSTVKRVLYHGLKGHSARKKPLLQKHHKKARLQFAKLHWEKDLCFWRHVLWSDGAKIELFGHNDQRYIWRTKGKAYKPKNTIPTVQYGGGSIMLWGCFAAGGTGPLHSIDGIMRKEHYVEILKQHLKTSARKLKLGHKWVFQMDHDPKHTAKLVKMCFKDNRVNVLEWPSQSPDLNPIENLWAELKKLVRARQPTNLTQLHQFCQEEWAKIPANYCEKLVEGYPKHLTKVIQFKSKAYKY

SEQ ID NO: 3 - protein, 340 aa, human
MGKNKELSQDLRSLIVEKHFDGNGYRRISRMLNVPVSTVGAIIRKWKKHKFTINRPRSGAPRKIPVRGVQRIIRRVLQEPRTTRAELQEDLASAGTIVSKKTISNALNHHGIHARSPRKTPLLNKKHVEARLKFAKQHLEKPVDYWETIVWSDESKIELFGSHSTHHVWRRNGTAHHPKNTIPTVKFGGGSIMVWGCFSARGTGRLHIIEGRMNGEMYRDILDKNLLPSTRKLKMKRGWTFQQDNDPKHKAKETMKWFQRKKIKLLEWPSQSPDLNPIENLWRELKIKVHKRGPRNLQDLKTVCVEEWARITPEQCRRLVSPYKRRLEAVITNKGFSTKY

SEQ ID NO: 4 - protein, 340 aa, human
MPRPKEIQEQLRKKVIEIYQSGKGYKAISKALGIQRTTVRAIIHKWRRHGTVVNLPRSGRPPKITPRAQRRLIQEVTKDPTTTSKELQASLASVKVSVHASTIRKRLGKNGLHGRVPRRKPLLSKKNIKARLNFSTTHLDDPQDFWDNILWTDETKVELFGRCVSKYIWRRRNTAFHKKNIIPTVKYGGGSVMVWGCFAASGPGRLAVIKGTMNSAVYQEILKENVRPSVRVLKLKRTWVLQQDNDPKHTSKSTTEWLKKNKMKTLEWPSQSPDLNPIEMLWYDLKKAVHARKPSNVTELGQFCKDEWAKIPPGRCKSLIARYRKRLVAVVAAKGGPTSY

SEQ ID NO: 5 - protein, 339 aa, human
MKTKELTKQVRDKVVEKYEAGLGYKKISRALNISLSTIKSIIRKWKEYGTTANLPRGGRPPKLKSRTRRKLIREATRRPMVTLEELQRSTAEVGESVHRTTISRLLHKSGLYGRVARRKPLLKGIHKKSRLEFARSHVGDTANMWKKVLWSDETKIELFGLNAKRYVWRKPNTAHHPEHTIPTVKHGGGSIMLWGCFSSAGTGKLVRIEGKMDGAKYREILEENLMQSAKDLRLGRRFIFQQDNDPKHTARATKEWFGLKNVNVLKWPSQSPDLNPIENLWQDLKIAVHRRSPSNLTELHLFCQEEWTNLSISRCAKLVETYPKRLAAVIAAKGGSTKY

SEQ ID NO: 6 - protein, 340 aa, Polyodon spathula
MARLSTATRHKVVILHQQGLSQAEISRQTGVSRCAVQALLKKHKETGNVEDRRRSGRPRKLTAADERHIMLTSLCNRKMSSSAISSELAENSGTEGHPSTVRRSLVRSGLHGRLAAKKPYLRRGNKAKRLNYARKHRNWGAKWQQVLWTDESKFEIFGCSRRQFVRRRAGERYTNECLQATVKHGGGSLQVWGCISANGVGDLVRINGLLNAEKYRQILIHHAIPSGRHLIGPKFILQHDNDPKHTAKVIKNYLQRKEEQGVLEVMVWPPQSPDLNIIESVWDYMKREKQLRLPKSTEELWLVLQDVWANLPAEFLQKLCASVPRRIDAVLKAKGGHTKY

SEQ ID NO: 7 - protein, 345 aa, human
MPGKRLAFEVTQLIYYNHQLGKSIPELVEIFSVSRKTVYNILNRAEKEGRLEPKSGGGCKTKINKRVDRLIMRKAIANPRISVRSLAQDIREECHLTVSHETVRQVILRHRYSSRVARKKPLLSEINIEKRHSFAVSMMDHAEEYWDDVIFCDETKMMLFYNDGPSRVWRKPLSALETQNIIPTIKFGKLSVMIWGCISSHGVGKLAFIESTMNAVQYLDILKTNLKASAEKFGLFSNNKPNFKFYQDNDPKHKEYNVRNWLLYNCGKVIDTPPQSPDLNPIENLWAYLKKKVAKRGPKTRQQLMAAIIAAWEKIPLEYDLKKLIHSMKKRLQLVAKANGGHTKY

SEQ ID NO: 8 - protein, 342 aa, human
MTREELSVSKRQDIIRLHGAQGKSYTEIAMLTNINRNTVARVIQRYKYEGRVSNLPRKGRPSVCTDRMRRAIKRLVDAEPEISAQSVAIVLNERHGIAISCETVRRYIHKFGYKAYNRRKKPQISPINRKRRLEFAKKYVNHPPEFWKKVLFTDESKFNIFGWDGTIKVWRPPGEGLNPKYTAKTVKHNGGGVLVWGCMAANGVGNLQVIDGIMDQYVYINILKQNLGPSLEKLGMSQDYWFQQDNDPKHTAFNSRLFLLYNTPHQLKSPPQSPDLNPIEHAWELLERKIWQTRIKNRVDLENKLKEAWITISEDYTQNLVNSMPERRLAEVIKMKGYATRY

SEQ ID NO: 9 - protein, 348 aa, human
MPGQRINENVIQLVYFHYHKGKCAKELAEMFSIKLRTIYNIINRAEKENRLELKHSGGRPAKLSRRDHSKILKQINENPQTSLRQLALDLKNDCNKTVSHETVRKVLKMHKYSSQIARKKPLLSAVNIQRRLNFSITNVNKPAEYWDDVIFCDETKIMLYYHDGPSKVWRKPNTALEQKNIIPTVKFGKLSVMVWGCISSKGVGELRIFNDVMTKEFYLDILKNELSRSAIKFGFVDPQNPSKQRYKLYQDNDPKHKSFLCRTWLLYNCSKVIDTPAQSPDLNPIENLWAFLKKRVGKRSPTNKNALIKAIQEEWIKIPEIYDLHNLIQSMSRRLRAVMDANGQYTKY

SEQ ID NO: 10 - protein, 343 aa, human
MVKSVGCKNLSLDVKKAIVAGFEQGIPTKMLALQIQRSPSTIWKVIKKYQTEKSVALRISPGRPRVTTHRMDRNILRSAREDPHRTATDIQMIISSPNEPVPSKRTVRRRLQQAGLHGRKPVKKPFISKKNRMARVAWAKAHLRWGRQEWAKHIWSDESKFNLFGSDGNSWVRRPVGSRYSPKYQCPTVKHGGGSVMVWGCFTSTSMGPLRRIQSIMDRFQYENIFETTMRPWALQNVGRGFVFQQDNDPKHTSLHVRSWFQRRHVHLLDWPSQSPDLNPIEHLWEELERRLGGIRASNADAKFNQLENAWKAIPMSVIHKLIDSMPRRCQAVIDANGYATKY

SEQ ID NO: 11 - protein, 341 aa, human
MVRGKPISKEIRVLIRDYFKSGKTLTEISKQLNLPKSSVHGVIQIFKKNGNIENNIANRGRTSAITPRDKRQLAKIVKADRRQSLRNLASKWSQTIGKTVKREWTRQQLKSIGYGFYKAKEKPLLTLRQKKKRLQWARERMSWTQRQWDTIIFSDEAKFDVSVGDTRKRVIRKRSETYHKDCLKRTTKFPASTMVWGCMSAKGLGKHLFIEGTVNAEKYINILQDSLLPSIPKLLDCGEFTFQQDGASSHTAKRTKNWLQYNQMEVLDWPSNSPDLSPIENIWWLMKNQLRNEPQRNISDLKIKLQEMWDSISQEHCKNLLSSMPKRVKCVMQAKGDVTQF

SEQ ID NO: 12 - protein, 337 aa, human
MGKRTTIEQRKLILEHFKIGYSYRQIAKMVNLSTTTVFNIIRRFVDENRIEDKGRKAPNKIFTEQEERRRIIRKIRENPKLSAPKLTQQVQDEMGKKCSVQTVRRVLHNHDFNARVPRKKPFISTKNKGTRMTFAKTHLDKDLEFWNTIIFEDESKFIIFGSDGRNYVRRQSNTELNPKNLKATVKHGGSVMVWACISAASVGNLVCIETTTDRNVDLSILKENLLQSAEKLGIRRYFRFYQDNDQTTTKHKSGLVPSWLIWNCPHMIIPAQSPDVNVINLWDLLENNIIRNHRSNLKNALLDEWSKISPETTRKLVSSMNNRLMEDIKAKGYHTKY

SEQ ID NO: 13 - protein, 339 aa, human
MPKTKELTVEARAGIVARFKAGTPAAKIAEIYQISRRTVYYLIKKFDTVGTLKNKKRSGRKPVLDQRQCRQILGVVAKNPSASPVKIALESKNTIGKQVSSSTIRRRLKEADFKTYVVRKTIEITPTNKTKRLRFALEYVKKPLDFWFNILWTDESAFQYQGSYSKHFMHLKNNQKHLAAQPTNRFGGGTVMFWGCLSYYGFGDLVPIEGTLNQNGYLLILNNHAFTSGNRLFPTTEWILQQDNAPCHKGRIPTKFLNDLNLAVLPWPPQSPDLNIIENVWAFIKNQRTIDKNRKREGAIIEIAEIWSKLTLEFAQTLVRSIPKRLQAVIDAKGGVTKY

SEQ ID NO: 14 - protein, 326 aa, human
MPRGSALSDTERAQDVMKLLNVSLHEMSRKISRSRHCIREYLKDPVSYGTSKRAPRRKALSVRDERNVIRAASNSCKTARDIRNELQLSASKRTILNVIKRSGVIVRQKLRPAPLLSADHKLKRLEFAKNMTNWSKVVFSDEKKFNLDGPDGCRYYWRDLRKEPMVFSRRNFGGGTVMVWGAFTEKKKLEIQFVSSKMNSTDYQNVLELELSKYLRHYSRKDFRFQQDNATIHVSNSTRDYFKLKKINLLDWPARSPDLNPIENLWGILVRIVYAQNKTYPTVASLKQGILDAWKSIPDNQLKSLVRSMEDRLIEIIRTQGNPINY

SEQ ID NO: 15 - protein, 311 aa, human
MPRGKELTPSLRSRICELKKQGYSYSQIHKHFPYIPLGTIKTTCRRAQRGAENTTLPRSGAPRKPHEEQRDQIYDTVITDPHVTTRDLLDSVDNVIKKRSLRYLLREMNKRKWIQKKRVALTPLQARKRLDWAIRYQGIDWRRVKWSDECMVRRGQGMRPIWTFLSPREPYAYRMFKKLGGRSCRQMFWAAFGHRSRTPLVPLVGKLNAIGIYELYSFILPWFLQSGDIFMHDNASVHTARIVKALLEELGVDLMTWPPYSPDLNPIENLWALMKAEIYRLHPELTHTEDTVATQHALVLAAMEAWDNIED

SEQ ID NO: 16 - protein, 348 aa, human
MEKKEFRVLIKYCFLKGKNTVEAKTWLDNEFPDSAPGKSTIIDWYAKFKRGEMSTEDGERSGRPKEVVTDENIKKIHKMILNDRKMKLIEIAEALKISKERVGHIIHQYLDMRKLCAKWVPRELTFDQKQQRVDDSERCLQLLTRNTPEFFRRYVTMDETWLHHYTPESNRQSAEWTATGEPSPKRGKTQKSAGKVMASVFFDAHGIIFIDYLEKGKTINSDYYMALLERLKVEIAAKRPHMKKKKVLFHQDNAPCHKSLRTMAKIHELGFELLPHPPYSPDLAPSDFFLFSDLKRMLAGKKFGCNEEVIAETEAYFEAKPKEYYQNGIKKLEGRYNRCIALEGNYVE

SEQ ID NO: 17 - protein, 345 aa, human
MSSFVPNKEQTRTVLIFCFHLKKTAAESHRMLVEAFGEQVPTVKTCERWFQRFKSGDFDVDDKEHGKPPKRYEDAELQALLDEDDAQTQKQLAEQLEVSQQAVSNRLREMGKIQKVGRWVPHELNERQMERRKNTCEILLSRYKRKSFLHRIVTGDEKWIFFVNPKRKKSYVDPGQPATSTARPNRFGKKTMLCVWWDQSGVIYYELLKPGETVNTARYQQQLINLNRALQRKRPEYQKRQHRVIFLHDNAPSHTARAVRDTLETLNWEVLPHAAYSPDLAPSDYHLFASMGHALAEQRFDSYESVKKWLDEWFAAKDDEFYWRGIHKLPERWEKCVASDGKYFE

SEQ ID NO: 18 - protein, 8 aa, artificial
  consensus sequence
  X (1)..(1): T, F, P, R
  X (2)..(2): I, T, N, R, K, Q, V
  X (3)..(3): K, N, L, R, Q
  Y (4)..(4): F, H, Y, L, S
  X (5)..(5): G, N, P, A, Q
  X (6)..(6): G, K, A or absent
  G (7)..(7): G
  X (8)..(8): S, or absent
XXXYXXGX

SEQ ID NO: 19 - protein, 9 aa, artificial
  consensus sequence
  X (1)..(1): Q, L, M, H, Y
  X (2)..(2): M, Q, H
  D (3)..(3): D
  X (4)..(4): N, H, G
  X (5)..(5): A, D
  Y (6)..(6): Q, P, S, T
  X (7)..(7): V, T, K
  Y (8)..(8): K, I, S, T, V, P, C
  H (9)..(9): H
XXDXXYXYH

SEQ ID NO: 20 - protein, 340 aa, artificial
  transposase with substitution H187V
MGKSKEISQDLRKRIVDLHKSGSSLGAISKRLAVPRSSVQTIVRKYKHHGTTQPSYRSGRRRVLSPRDERTLVRKVQINPRTTAKDLVKMLEETGTKVSISTVKRVLYRHNLKGHSARKKPLLQNRHKKARLRFATAHGDKDRTFWRNVLWSDETKIELFGHNDHRYVWRKKGEACKPKNTIPTVKVGGGSIMLWGCFAAGGTGALHKIDGIMDAVQYVDILKQHLKTSVRKLKLGRKWVFQHDNDPKHTSKVVAKWLKDNKVKVLEWPSQSPDLNPIENLWAELKKRVRARRPTNLTQLHQLCQEEWAKIHPNYCGKLVEGYPKRLTQVKQFKGNATKY

SEQ ID NO: 21 - protein, 340 aa, artificial
  transposase with substitution P247R
MGKSKEISQDLRKRIVDLHKSGSSLGAISKRLAVPRSSVQTIVRKYKHHGTTQPSYRSGRRRVLSPRDERTLVRKVQINPRTTAKDLVKMLEETGTKVSISTVKRVLYRHNLKGHSARKKPLLQNRHKKARLRFATAHGDKDRTFWRNVLWSDETKIELFGHNDHRYVWRKKGEACKPKNTIPTVKHGGGSIMLWGCFAAGGTGALHKIDGIMDAVQYVDILKQHLKTSVRKLKLGRKWVFQHDNDRKHTSKVVAKWLKDNKVKVLEWPSQSPDLNPIENLWAELKKRVRARRPTNLTQLHQLCQEEWAKIHPNYCGKLVEGYPKRLTQVKQFKGNATKY

SEQ ID NO: 22 - protein, 340 aa, artificial
  transposase with substitution K248R
MGKSKEISQDLRKRIVDLHKSGSSLGAISKRLAVPRSSVQTIVRKYKHHGTTQPSYRSGRRRVLSPRDERTLVRKVQINPRTTAKDLVKMLEETGTKVSISTVKRVLYRHNLKGHSARKKPLLQNRHKKARLRFATAHGDKDRTFWRNVLWSDETKIELFGHNDHRYVWRKKGEACKPKNTIPTVKHGGGSIMLWGCFAAGGTGALHKIDGIMDAVQYVDILKQHLKTSVRKLKLGRKWVFQHDNDPRHTSKVVAKWLKDNKVKVLEWPSQSPDLNPIENLWAELKKRVRARRPTNLTQLHQLCQEEWAKIHPNYCGKLVEGYPKRLTQVKQFKGNATKY